European Patent Specification EP 3 775 178 B1, published August 6, 2025. Title: NOVEL NADH-DEPENDENT ENZYME MUTANTS TO CONVERT ACETONE INTO ISOPROPANOL. Applicant: Braskem S.A. The sequence listing filed with the application follows.

SEQUENCE LISTING (27 sequences)

SEQ ID NO: 1 - DNA, 1056 bp, Clostridium beijerinckii
atgaaagggtttgccatgttaggtatcaataaactgggctggattgaaaaagagcgcccggtggcgggttcatacgatgcaattgttcgtccgctggccgtcagtccgtgcaccagcgacatccatacagtctttgaaggtgccctgggtgatcggaaaaacatgattctgggccatgaagccgtaggcgaagtagtggaagtgggcagcgaggtaaaggatttcaaaccgggtgatcgcgtaattgttccttgcacgaccccagattggcgctcactggaagttcaggctggttttcagcagcatagtaacggtatgttagcaggctggaagtttagcaattttaaagacggggtgttcggggagtattttcatgtcaacgatgcggacatgaatctggctattttacctaaagatatgccgctggagaacgcagtgatgattaccgacatgatgacgacaggctttcacggtgcagaactggctgacatccaaatgggctccagtgtggtggttatcggtattggtgcggtcgggctgatgggtatcgcgggcgcgaaattacggggcgctggtcgcatcatcggtgtcggcagccgtccaatttgcgttgaagcagctaaattctatggtgccacggacattctgaactataaaaatggtcacatcgtcgatcaggtgatgaaactgaccaatggcaaaggtgtggaccgcgtgatcatggcgggcggcggctcagagactttatctcaagcggtgtctatggttaaacctgggggcatcatttctaatattaactatcatggctccggcgacgcattactgatcccgcgtgttgaatggggctgtgggatggcccacaaaaccattaaaggggggttatgtccgggtggtcgcctgcgtgccgaaatgctgcgtgacatggtggtttacaaccgtgtggatctgtccaaactggtaactcacgtataccacggtttcgatcacattgaagaggcgctgctgctgatgaaggataagccaaaggatctgattaaggcggttgttatcctgtaa

SEQ ID NO: 2 - protein, 351 aa, Clostridium beijerinckii
MKGFAMLGINKLGWIEKERPVAGSYDAIVRPLAVSPCTSDIHTVFEGALGDRKNMILGHEAVGEVVEVGSEVKDFKPGDRVIVPCTTPDWRSLEVQAGFQQHSNGMLAGWKFSNFKDGVFGEYFHVNDADMNLAILPKDMPLENAVMITDMMTTGFHGAELADIQMGSSVVVIGIGAVGLMGIAGAKLRGAGRIIGVGSRPICVEAAKFYGATDILNYKNGHIVDQVMKLTNGKGVDRVIMAGGGSETLSQAVSMVKPGGIISNINYHGSGDALLIPRVEWGCGMAHKTIKGGLCPGGRLRAEMLRDMVVYNRVDLSKLVTHVYHGFDHIEEALLLMKDKPKDLIKAVVIL

SEQ ID NO: 3 - protein, 351 aa, Artificial Sequence
  Modified ADH from Clostridium beijerinckii
MKGFAMLGINKLGWIEKERPVAGSYDAIVRPLAVSPCTSDIHTVFEGALGDRKNMILGHEAVGEVVEVGSEVKDFKPGDRVIVPCTTPDWRSLEVQAGFQQHSNGMLAGWKFSNFKDGVFGEYFHVNDADMNLAILPKDMPLENAVMITDMMTTGFHGAELADIQMGSSVVVCGIGAVGLMGIAGAKLRGAGRIIGVESRPICVEAAKFYGATDILNYKNGHIVDQVMKLTNGKGVDRVIMAGGGSETLSQAVSMVKPGGIISNINYHGSGDALLIPRVEWGCGMAHKTIKGGLCPGGRLRAEMLRDMVVYNRVDLSKLVTHVYHGFDHIEEALLLMKDKPKDLIKAVVIL

SEQ ID NO: 4 - protein, 351 aa, Artificial Sequence
  Modified ADH from Clostridium beijerinckii
MKGFAMLGINKLGWIEKERPVAGSYDAIVRPLAVSPCTSDIHTVFEGALGDRKNMILGHEAVGEVVEVGSEVKDFKPGDRVIVPCTTPDWRSLEVQAGFQQHSNGMLAGWKFSNFKDGVFGEYFHVNDADMNLAILPKDMPLENAVMITDMMTTGFHGAELADIQMGSSVVVIGIGAVGLMGIAGAKLRGAGRIIGVESRPICVEAAKFYGATDILNYKNGHIVDQVMKLTNGKGVDRVIMAGGGSETLSQAVSMVKPGGIISNINYHGSGDALLIPRVEWGCGMAHKTIKGGLCPGGRLRAEMLRDMVVYNRVDLSKLVTHVYHGFDHIEEALLLMKDKPKDLIKAVVIL

SEQ ID NO: 5 - protein, 351 aa, Artificial Sequence
  Modified ADH from Clostridium beijerinckii
MKGFAMLGINKLGWIEKERPVAGSYDAIVRPLAVSPCTSDIHTVFEGALGDRKNMILGHEAVGEVVEVGSEVKDFKPGDRVIVPCTTPDWRSLEVQAGFQQHSNGMLAGWKFSNFKDGVFGEYFHVNDADMNLAILPKDMPLENAVMITDMMTTGFHGAELADIQMGSSVVVIGIGAVGLMGIAGAKLRGAGRIIGVESRPICVEAAKFYGATDILNFKNGHIVDQVMKLTNGKGVDRVIMAGGGSETLSQAVSMVKPGGIISNINYHGSGDALLIPRVEWGCGMAHKTIKGGLCPGGRLRAEMLRDMVVYNRVDLSKLVTHVYHGFDHIEEALLLMKDKPKDLIKAVVIL

SEQ ID NO: 6 - protein, 351 aa, Artificial Sequence
  Modified ADH from Clostridium beijerinckii
MKGFAMLGINKLGWIEKERPVAGSYDAIVRPLAVSPCTSDIHTVFEGALGDRKNMILGHEAVGEVVEVGSEVKDFKPGDRVIVPCTTPDWRSLEVQAGFQQHSNGMLAGWKFSNFKDGVFGEYFHVNDADMNLAILPKDMPLENAVMITDMMTTGFHGAELADIQMGSSVVVIGIGAVGLMGIAGAKLRGAGRIIGVESRPICVEAAKFYGATDILNPKNGHIVDQVMKLTNGKGVDRVIMAGGGSETLSQAVSMVKPGGIISNINYHGSGDALLIPRVEWGCGMAHKTIKGGLCPGGRLRAEMLRDMVVYNRVDLSKLVTHVYHGFDHIEEALLLMKDKPKDLIKAVVIL

SEQ ID NO: 7 - protein, 351 aa, Artificial Sequence
  Modified ADH from Clostridium beijerinckii
MKGFAMLGINKLGWIEKERPVAGSYDAIVRPLAVSPCTSDIHTVFEGALGDRKNMILGHEAVGEVVEVGSEVKDFKPGDRVIVPCTTPDWRSLEVQAGFQQHSNGMLAGWKFSNFKDGVFGEYFHVNDADMNLAILPKDMPLENAVMITDMMTTGFHGAELADIQMGSSVVVIGIGAVGLMGIAGAKLRGAGRIIGVESRPICVEAAKFYGATDILNAKNGHIVDQVMKLTNGKGVDRVIMAGGGSETLSQAVSMVKPGGIISNINYHGSGDALLIPRVEWGCGMAHKTIKGGLCPGGRLRAEMLRDMVVYNRVDLSKLVTHVYHGFDHIEEALLLMKDKPKDLIKAVVIL

SEQ ID NO: 8 - protein, 351 aa, Artificial Sequence
  Modified ADH from Clostridium beijerinckii
MKGFAMLGINKLGWIEKERPVAGSYDAIVRPLAVSPCTSDIHTVFEGALGDRKNMILGHEAVGEVVEVGSEVKDFKPGDRVIVPCTTPDWRSLEVQAGFQQHSNGMLAGWKFSNFKDGVFGEYFHVNDADMNLAILPKDMPLENAVMITDMMTTGFHGAELADIQMGSSVVVIGIGAVGLMGIAGAKLRGAGRIIGVESRPICVEAAKFYGATDILNWKNGHIVDQVMKLTNGKGVDRVIMAGGGSETLSQAVSMVKPGGIISNINYHGSGDALLIPRVEWGCGMAHKTIKGGLCPGGRLRAEMLRDMVVYNRVDLSKLVTHVYHGFDHIEEALLLMKDKPKDLIKAVVIL

SEQ ID NO: 9 - protein, 351 aa, Artificial Sequence
  Modified ADH from Clostridium beijerinckii
MKGFAMLGINKLGWIEKERPVAGSYDAIVRPLAVSPCTSDIHTVFEGALGDRKNMILGHEAVGEVVEVGSEVKDFKPGDRVIVPCTTPDWRSLEVQAGFQQHSNGMLAGWKFSNFKDGVFGEYFHVNDADMNLAILPKDMPLENAVMITDMMTTGFHGAELADIQMGSSVVVIGIGAVGLMGIAGAKLRGAGRIIGVEDRPICVEAAKFYGATDILNYKNGHIVDQVMKLTNGKGVDRVIMAGGGSETLSQAVSMVKPGGIISNINYHGSGDALLIPRVEWGCGMAHKTIKGGLCPGGRLRAEMLRDMVVYNRVDLSKLVTHVYHGFDHIEEALLLMKDKPKDLIKAVVIL

SEQ ID NO: 10 - protein, 351 aa, Artificial Sequence
  Modified ADH from Clostridium beijerinckii
MKGFAMLGINKLGWIEKERPVAGSYDAIVRPLAVSPCTSDIHTVFEGALGDRKNMILGHEAVGEVVEVGSEVKDFKPGDRVIVPCTTPDWRSLEVQAGFQQHSNGMLAGWKFSNFKDGVFGEYFHVNDADMNLAILPKDMPLENAVMITDMMTTGFHGAELADIQMGSSVVVIGIGAVGLMGIAGAKLRGAGRIIGVEIRPICVEAAKFYGATDILNYKNGHIVDQVMKLTNGKGVDRVIMAGGGSETLSQAVSMVKPGGIISNINYHGSGDALLIPRVEWGCGMAHKTIKGGLCPGGRLRAEMLRDMVVYNRVDLSKLVTHVYHGFDHIEEALLLMKDKPKDLIKAVVIL

SEQ ID NO: 11 - protein, 351 aa, Artificial Sequence; identical to SEQ ID NO: 4
  Modified ADH from Clostridium beijerinckii

SEQ ID NO: 12 - protein, 351 aa, Artificial Sequence
  Modified ADH from Clostridium beijerinckii
MKGFAMLGINKLGWIEKERPVAGSYDAIVRPLAVSPCTSDIHTVFEGALGDRKNMILGHEAVGEVVEVGSEVKDFKPGDRVIVPCTTPDWRSLEVQAGFQQHSNGMLAGWKFSNFKDGVFGEYFHVNDADMNLAILPKDMPLENAVMITDMMTTGFHGAELADIQMGSSVVVIGIGAVGLMGIAGAKLRGAGRIIGVESRPICVEAAKFYGATDILNYKNGHIVDQVMKLTNGKGVDRVIMAGLGSETLSQAVSMVKPGGIISNINYHGSGDALLIPRVEWGCGMAHKTIKGGLCPGGRLRAEMLRDMVVYNRVDLSKLVTHVYHGFDHIEEALLLMKDKPKDLIKAVVIL

SEQ ID NO: 13 - protein, 351 aa, Artificial Sequence
  Modified ADH from Clostridium beijerinckii
MKGFAMLGINKLGWIEKERPVAGSYDAIVRPLAVSPCTSDIHTVFEGALGDRKNMILGHEAVGEVVEVGSEVKDFKPGDRVIVPCTTPDWRSLEVQAGFQQHSNGMLAGWKFSNFKDGVFGEYFHVNDADMNLAILPKDMPLENAVMITDMMTTGFHGAELADIQMGSSVVVIGIGAVGLMGIAGAKLRGAGRIIGVESRPICVEAAKFYGATDILNYKNGHIVDQVMKLTNGKGVDRVIMAGCGSETLSQAVSMVKPGGIISNINYHGSGDALLIPRVEWGCGMAHKTIKGGLCPGGRLRAEMLRDMVVYNRVDLSKLVTHVYHGFDHIEEALLLMKDKPKDLIKAVVIL

SEQ ID NO: 14 - protein, 351 aa, Artificial Sequence
  Modified ADH from Clostridium beijerinckii
MKGFAMLGINKLGWIEKERPVAGSYDAIVRPLAVSPCTSDIHTVFEGALGDRKNMILGHEAVGEVVEVGSEVKDFKPGDRVIVPCTTPDWRSLEVQAGFQQHSNGMLAGWKFSNFKDGVFGEYFHVNDADMNLAILPKDMPLENAVMITDMMTTGFHGAELADIQMGSSVVVIGIGAVGLMGIAGAKLRGAGRIIGVESRPICVEAAKFYGATDILNYKNGHIVDQVMKLTNGKGVDRVIMAGGGSDTLSQAVSMVKPGGIISNINYHGSGDALLIPRVEWGCGMAHKTIKGGLCPGGRLRAEMLRDMVVYNRVDLSKLVTHVYHGFDHIEEALLLMKDKPKDLIKAVVIL

SEQ ID NO: 15 - protein, 351 aa, Artificial Sequence
  Modified ADH from Clostridium beijerinckii
MKGFAMLGINKLGWIEKERPVAGSYDAIVRPLAVSPCTSDIHTVFEGALGDRKNMILGHEAVGEVVEVGSEVKDFKPGDRVIVPCTTPDWRSLEVQAGFQQHSNGMLAGWKFSNFKDGVFGEYFHVNDADMNLAILPKDMPLENAVMITDMMTTGFHGAELADIQMGSSVVVIGIGAVGLMGIAGAKLRGAGRIIGVESRPICVEAAKFYGATDILNYKNGHIVDQVMKLTNGKGVDRVIMAGGGSNTLSQAVSMVKPGGIISNINYHGSGDALLIPRVEWGCGMAHKTIKGGLCPGGRLRAEMLRDMVVYNRVDLSKLVTHVYHGFDHIEEALLLMKDKPKDLIKAVVIL

SEQ ID NO: 16 - protein, 351 aa, Artificial Sequence
  Modified ADH from Clostridium beijerinckii
MKGFAMLGINKLGWIEKERPVAGSYDAIVRPLAVSPCTSDIHTVFEGALGDRKNMILGHEAVGEVVEVGSEVKDFKPGDRVIVPCTTPDWRSLEVQAGFQQHSNGMLAGWKFSNFKDGVFGEYFHVNDADMNLAILPKDMPLENAVMITDMMTTGFHGAELADIQMGSSVVVIGIGAVGLMGIAGAKLRGAGRIIGVESRPICVEAAKFYGATDILNYKNGHIVDQVMKLTNGKGVDRVIMAGGGSQTLSQAVSMVKPGGIISNINYHGSGDALLIPRVEWGCGMAHKTIKGGLCPGGRLRAEMLRDMVVYNRVDLSKLVTHVYHGFDHIEEALLLMKDKPKDLIKAVVIL

SEQ ID NO: 17 - protein, 351 aa, Artificial Sequence
  Modified ADH from Clostridium beijerinckii
MKGFAMLGINKLGWIEKERPVAGSYDAIVRPLAVSPCTSDIHTVFEGALGDRKNMILGHEAVGEVVEVGSEVKDFKPGDRVIVPCTTPDWRSLEVQAGFQQHSNGMLAGWKFSNFKDGVFGEYFHVNDADMNLAILPKDMPLENAVMITDMMTTGFHGAELADIQMGSSVVVIGIGAVGLMGIAGAKLRGAGRIIGVDSRPICVEAAKFYGATDILNYKNGHIVDQVMKLTNGKGVDRVIMAGGGSETLSQAVSMVKPGGIISNINYHGSGDALLIPRVEWGCGMAHKTIKGGLCPGGRLRAEMLRDMVVYNRVDLSKLVTHVYHGFDHIEEALLLMKDKPKDLIKAVVIL

SEQ ID NO: 18 - protein, 351 aa, Artificial Sequence
  Modified ADH from Clostridium beijerinckii
MKGFAMLGINKLGWIEKERPVAGSYDAIVRPLAVSPCTSDIHTVFEGALGDRKNMILGHEAVGEVVEVGSEVKDFKPGDRVIVPCTTPDWRSLEVQAGFQQHSNGMLAGWKFSNFKDGVFGEYFHVNDADMNLAILPKDMPLENAVMITDMMTTGFHGAELADIQMGSSVVVIGIGAVGLMGIAGAKLRGAGRIIGVDIRPICVEAAKFYGATDILNYKNGHIVDQVMKLTNGKGVDRVIMAGGGSETLSQAVSMVKPGGIISNINYHGSGDALLIPRVEWGCGMAHKTIKGGLCPGGRLRAEMLRDMVVYNRVDLSKLVTHVYHGFDHIEEALLLMKDKPKDLIKAVVIL

SEQ ID NO: 19 - protein, 351 aa, Artificial Sequence
  Modified ADH from Clostridium beijerinckii
MKGFAMLGINKLGWIEKERPVAGSYDAIVRPLAVSPCTSDIHTVFEGALGDRKNMILGHEAVGEVVEVGSEVKDFKPGDRVIVPCTTPDWRSLEVQAGFQQHSNGMLAGWKFSNFKDGVFGEYFHVNDADMNLAILPKDMPLENAVMITDMMTTGFHGAELADIQMGSSVVVIGIGAVGLMGIAGAKLRGAGRIIGVDGRPICVEAAKFYGATDILNYKNGHIVDQVMKLTNGKGVDRVIMAGGGSETLSQAVSMVKPGGIISNINYHGSGDALLIPRVEWGCGMAHKTIKGGLCPGGRLRAEMLRDMVVYNRVDLSKLVTHVYHGFDHIEEALLLMKDKPKDLIKAVVIL

SEQ ID NO: 20 - protein, 351 aa, Artificial Sequence
  Modified ADH from Clostridium beijerinckii
MKGFAMLGINKLGWIEKERPVAGSYDAIVRPLAVSPCTSDIHTVFEGALGDRKNMILGHEAVGEVVEVGSEVKDFKPGDRVIVPCTTPDWRSLEVQAGFQQHSNGMLAGWKFSNFKDGVFGEYFHVNDADMNLAILPKDMPLENAVMITDMMTTGFHGAELADIQMGSSVVVIGIGAVGLMGIAGAKLRGAGRIIGVDSRPICVEAAKFYGATDILNFKNGHIVDQVMKLTNGKGVDRVIMAGGGSETLSQAVSMVKPGGIISNINYHGSGDALLIPRVEWGCGMAHKTIKGGLCPGGRLRAEMLRDMVVYNRVDLSKLVTHVYHGFDHIEEALLLMKDKPKDLIKAVVIL

SEQ ID NO: 21 - protein, 351 aa, Artificial Sequence
  Modified ADH from Clostridium beijerinckii
MKGFAMLGINKLGWIEKERPVAGSYDAIVRPLAVSPCTSDIHTVFEGALGDRKNMILGHEAVGEVVEVGSEVKDFKPGDRVIVPCTTPDWRSLEVQAGFQQHSNGMLAGWKFSNFKDGVFGEYFHVNDADMNLAILPKDMPLENAVMITDMMTTGFHGAELADIQMGSSVVVIGIGAVGLMGIAGAKLRGAGRIIGVDSRPICVEAAKFYGATDILNPKNGHIVDQVMKLTNGKGVDRVIMAGGGSETLSQAVSMVKPGGIISNINYHGSGDALLIPRVEWGCGMAHKTIKGGLCPGGRLRAEMLRDMVVYNRVDLSKLVTHVYHGFDHIEEALLLMKDKPKDLIKAVVIL

SEQ ID NO: 22 - protein, 351 aa, Artificial Sequence
  Modified ADH from Clostridium beijerinckii
MKGFAMLGINKLGWIEKERPVAGSYDAIVRPLAVSPCTSDIHTVFEGALGDRKNMILGHEAVGEVVEVGSEVKDFKPGDRVIVPCTTPDWRSLEVQAGFQQHSNGMLAGWKFSNFKDGVFGEYFHVNDADMNLAILPKDMPLENAVMITDMMTTGFHGAELADIQMGSSVVVIGIGAVGLMGIAGAKLRGAGRIIGVDSRPICVEAAKFYGATDILNWKNGHIVDQVMKLTNGKGVDRVIMAGGGSETLSQAVSMVKPGGIISNINYHGSGDALLIPRVEWGCGMAHKTIKGGLCPGGRLRAEMLRDMVVYNRVDLSKLVTHVYHGFDHIEEALLLMKDKPKDLIKAVVIL

SEQ ID NO: 23 - protein, 351 aa, Artificial Sequence
  Modified ADH from Clostridium beijerinckii
MKGFAMLGINKLGWIEKERPVAGSYDAIVRPLAVSPCTSDIHTVFEGALGDRKNMILGHEAVGEVVEVGSEVKDFKPGDRVIVPCTTPDWRSLEVQAGFQQHSNGMLAGWKFSNFKDGVFGEYFHVNDADMNLAILPKDMPLENAVMITDMMTTGFHGAELADIQMGSSVVVIGIGAVGLMGIAGAKLRGAGRIIGVDSRPICVEAAKFYGATDILNAKNGHIVDQVMKLTNGKGVDRVIMAGGGSETLSQAVSMVKPGGIISNINYHGSGDALLIPRVEWGCGMAHKTIKGGLCPGGRLRAEMLRDMVVYNRVDLSKLVTHVYHGFDHIEEALLLMKDKPKDLIKAVVIL

SEQ ID NO: 24 - protein, 351 aa, Artificial Sequence
  Modified ADH from Clostridium beijerinckii
MKGFAMLGINKLGWIEKERPVAGSYDAIVRPLAVSPCTSDIHTVFEGALGDRKNMILGHEAVGEVVEVGSEVKDFKPGDRVIVPCTTPDWRSLEVQAGFQQHSNGMLAGWKFSNFKDGVFGEYFHVNDADMNLAILPKDMPLENAVMITDMMTTGFHGAELADIQMGSSVVVIGIGAVGLMGIAGAKLRGAGRIIGVDVREICVEAAKFYGATDILNAKNGHIVDQVMKLTNGKGVDRVIMAGGGSETLSQAVSMVKPGGIISNINYHGSGDALLIPRVEWGCGMAHKTIKGGLCPGGRLRAEMLRDMVVYNRVDLSKLVTHVYHGFDHIEEALLLMKDKPKDLIKAVVIL

SEQ ID NO: 25 - protein, 351 aa, Artificial Sequence
  Modified ADH from Clostridium beijerinckii
MKGFAMLGINKLGWIEKERPVAGSYDAIVRPLAVSPCTSDIHTVFEGALGDRKNMILGHEAVGEVVEVGSEVKDFKPGDRVIVPCTTPDWRSLEVQAGFQQHSNGMLAGWKFSNFKDGVFGEYFHVNDADMNLAILPKDMPLENAVMITDMMTTGFHGAELADIQMGSSVVVIGIGAVGLMGIAGAKLRGAGRIIGVDVRRICVEAAKFYGATDILNYKNGHIVDQVMKLTNGKGVDRVIMAGGGSETLSQAVSMVKPGGIISNINYHGSGDALLIPRVEWGCGMAHKTIKGGLCPGGRLRAEMLRDMVVYNRVDLSKLVTHVYHGFDHIEEALLLMKDKPKDLIKAVVIL

SEQ ID NO: 26 - protein, 351 aa, Artificial Sequence
  Modified ADH from Clostridium beijerinckii
MKGFAMLGINKLGWIEKERPVAGSYDAIVRPLAVSPCTSDIHTVFEGALGDRKNMILGHEAVGEVVEVGSEVKDFKPGDRVIVPCTTPDWRSLEVQAGFQQHSNGMLAGWKFSNFKDGVFGEYFHVNDADMNLAILPKDMPLENAVMITDMMTTGFHGAELADIQMGSSVVVIGIGAVGLMGIAGAKLRGAGRIIGVLDRPICVEAAKFYGATDILNYKNGHIVDQVMKLTNGKGVDRVIMAGGGSETLSQAVSMVKPGGIISNINYHGSGDALLIPRVEWGCGMAHKTIKGGLCPGGRLRAEMLRDMVVYNRVDLSKLVTHVYHGFDHIEEALLLMKDKPKDLIKAVVIL

SEQ ID NO: 27 - protein, 351 aa, Artificial Sequence
  Modified ADH from Clostridium beijerinckii
MKGFAMLGINKLGWIEKERPVAGSYDAIVRPLAVSPCTSDIHTVFEGALGDRKNMILGHEAVGEVVEVGSEVKDFKPGDRVIVPCTTPDWRSLEVQAGFQQHSNGMLAGWKFSNFKDGVFGEYFHVNDADMNLAILPKDMPLENAVMITDMMTTGFHGAELADIQMGSSVVVIGRGAVGLMGIAGAKLRGAGRIIGVLDRPICVEAAKFYGATDILNDKNGHIVDQVMKLTNGKGVDRVIMAGGGSETLSQAVSMVKPGGIISNINYHGSGDALLIPRVEWGCGMAHKTIKGGLCPGGRLRAEMLRDMVVYNRVDLSKLVTHVYHGFDHIEEALLLMKDKPKDLIKAVVIL